European Patent Application EP 4 356 919 A1, published April 24, 2024. Title: Compositions for improving drug sensitivity of antibacterial agents to methicillin-resistant yellow staphylococcus (MRSA), compositions for treating or preventing MRSA infections, and compositions for reducing the pathogenicity of MRSA. Applicant: INCORPORATED EDUCATIONAL INSTITUTION RAKUNO GAKUEN. The sequence listing filed with the application follows.

SEQUENCE LISTING (4 sequences)

SEQ ID NO: 1 - DNA, 21 bp, synthetic construct
  misc_feature 1..21: note = femA forward primer
  source 1..21: mol_type = other DNA
caaagccatcattctcacggg

SEQ ID NO: 2 - DNA, 23 bp, synthetic construct
  misc_feature 1..23: note = femA reverse primer
  source 1..23: mol_type = other DNA
cagaggggaaatagaaaaactgc

SEQ ID NO: 3 - DNA, 22 bp, synthetic construct
  misc_feature 1..22: note = mgrA forward primer
  source 1..22: mol_type = other DNA
gctcaaagacaagttaatcgct

SEQ ID NO: 4 - DNA, 25 bp, synthetic construct
  misc_feature 1..25: note = mgrA reverse primer
  source 1..25: mol_type = other DNA
atcaaatgcatgaatgactttacct